European Patent Specification EP 3 288 578 B1, published March 15, 2023. Title: Compositions for Colon Cleansing and the Treatment of Gastrointestinal Disorders. Applicant: Ironwood Pharmaceuticals, Inc. The sequence listing filed with the application follows.

SEQUENCE LISTING (94 sequences)

SEQ ID NO: 1 - protein, 21 aa, Artificial Sequence
  Synthetically generated peptide
  VARIANT (1)..(1): Xaa1 is glutamic acid wherein the side chain carboxylic acid forms the peptide linkage or is absent
  VARIANT (2)..(2): Xaa2 is lysine wherein the side chain amine forms the peptide linkage, Asn or is absent
  VARIANT (3)..(3): Xaa3 is Asn, Ser or is absent
  VARIANT (4)..(4): Xaa4 is Ser or is absent
  VARIANT (5)..(5): Xaa5 is Ser, Asn, Ile, glutamic acid wherein the side chain carboxylic acid forms the peptide linkage or is absent
  VARIANT (6)..(6): Xaa6 is Tyr, Asp, 4-fluorophenylalanine ((4-F)Phe), lysine wherein the side chain amine forms the peptide linkage or is absent
  VARIANT (7)..(7): Xaa7 is Cys, cystathionine (Cth), allylglycine (Ag), allylglycine with a reduced dicarba bond (Hag), or Asp
  MISC_FEATURE (7)..(12): covalent bond between Xaa7 and Xaa12
  VARIANT (8)..(8): Xaa8 is Cys, cystathionine (Cth), penicillamine (Pen), or allylglycine (Ag)
  MISC_FEATURE (8)..(16): covalent bond between Xaa8 and Xaa16
  VARIANT (9)..(9): Xaa9 is Glu, Asp, Ser, Thr, or Gln
  VARIANT (10)..(10): Xaa10 is Leu, cyclohexylalanine (Cha), Phe, or 4-fluorophenylalanine ((4-F)Phe)
  VARIANT (11)..(11): Xaa11 is Cys, allylglycine (Ag), or penicillamine (Pen)
  MISC_FEATURE (11)..(19): covalent bond between Xaa11 and Xaa19
  VARIANT (12)..(12): Xaa12 is Cys, allylglycine (Ag), allylglycine with a reduced dicarba bond (Hag), cystathionine (Cth), di-aminopropionic acid (Dpr), or Val
  VARIANT (13)..(13): Xaa13 is Asn or Leu
  VARIANT (14)..(14): Xaa14 is Pro, Val, sarcosine (Sar), Leu, or Hydroxyproline (OH-Pro)
  VARIANT (16)..(16): Xaa16 is Cys, allylglycine (Ag), penicillamine (Pen) or cystathionine (Cth)
  VARIANT (17)..(17): Xaa17 is Tyr, Thr, cyclohexylalanine (Cha), 4-fluorophenylalanine ((4-F)Phe), Phe, Ser, or Ala
  VARIANT (19)..(19): Xaa19 is Cys, Ag or Pen
  VARIANT (20)..(20): Xaa20 is Tyr, Leu, 4-fluorophenylalanine ((4-F)Phe), cyclohexylalanine (Cha), D-Tyr, N-Methyl Tyr (Nme-Tyr) or is absent
  VARIANT (21)..(21): Xaa21 is absent or Asn
XXXXXXXXXXXXXXAXXGXXX

SEQ ID NO: 2 - protein, 14 aa, Artificial Sequence
  Synthetically generated peptide
  MOD_RES (1)..(1): allylglycine
  MOD_RES (6)..(6): allylglycine
  MOD_RES (14)..(14): AMIDATION
GCELCGNPACTGCY

SEQ ID NO: 3 - protein, 20 aa, Artificial Sequence
  Synthetically generated peptide
  MOD_RES (1)..(1): N-terminus capped with C12 alkyl carboxylic acid
  MOD_RES (1)..(1): glutamic acid wherein the side chain carboxylic acid forms the peptide linkage
  MOD_RES (2)..(2): lysine wherein the side chain amine forms the peptide linkage
  MOD_RES (20)..(20): AMIDATION
EKNSSYCCELCCNPACTGCY

SEQ ID NO: 4 - protein, 20 aa, Artificial Sequence
  Synthetically generated peptide
  MOD_RES (1)..(1): N-terminus capped with C16 alkyl carboxylic acid
  MOD_RES (1)..(1): glutamic acid wherein the side chain carboxylic acid forms the peptide linkage
  MOD_RES (2)..(2): lysine wherein the side chain amine forms the peptide linkage
  MOD_RES (20)..(20): AMIDATION
EKNSSYCCELCCNPACTGCY

SEQ ID NO: 5 - protein, 20 aa, Artificial Sequence
  Synthetically generated peptide
  MOD_RES (1)..(1): N-terminus capped with C12 alkyl carboxylic acid
  MOD_RES (1)..(1): glutamic acid wherein the side chain carboxylic acid forms the peptide linkage
  MOD_RES (2)..(2): lysine wherein the side chain amine forms the peptide linkage
EKNSSYCCELCCNPACTGCY

SEQ ID NO: 6 - protein, 20 aa, Artificial Sequence
  Synthetically generated peptide
  MOD_RES (1)..(1): N-terminus capped with C14 alkyl carboxylic acid
  MOD_RES (1)..(1): glutamic acid wherein the side chain carboxylic acid forms the peptide linkage
  MOD_RES (2)..(2): lysine wherein the side chain amine forms the peptide linkage
EKNSSYCCELCCNPACTGCY

SEQ ID NO: 7 - protein, 20 aa, Artificial Sequence
  Synthetically generated peptide
  MOD_RES (1)..(1): N-terminus capped with C16 alkyl carboxylic acid
  MOD_RES (1)..(1): glutamic acid wherein the side chain carboxylic acid forms the peptide linkage
  MOD_RES (2)..(2): lysine wherein the side chain amine forms the peptide linkage
EKNSSYCCELCCNPACTGCY

SEQ ID NO: 8 - protein, 14 aa, Artificial Sequence
  Synthetically generated peptide
  MOD_RES (2)..(2): allylglycine
  MOD_RES (10)..(10): allylglycine
  MOD_RES (14)..(14): AMIDATION
CGELCCNPAGTGCY

SEQ ID NO: 9 - protein, 16 aa, Artificial Sequence
  Synthetically generated peptide
  MOD_RES (4)..(4): allylglycine
  MOD_RES (12)..(12): allylglycine
  MOD_RES (16)..(16): AMIDATION
NDDGELCVNVAGTGCL

SEQ ID NO: 10 - protein, 16 aa, Artificial Sequence
  Synthetically generated peptide
  MOD_RES (7)..(7): allylglycine
  MOD_RES (15)..(15): allylglycine
  MOD_RES (16)..(16): AMIDATION
NDDCELGVNVACTGGL

SEQ ID NO: 11 - protein, 20 aa, Artificial Sequence
  Synthetically generated peptide
  MOD_RES (1)..(1): N-terminus capped with C18 alkyl carboxylic acid
  MOD_RES (1)..(1): glutamic acid wherein the side chain carboxylic acid forms the peptide linkage
  MOD_RES (2)..(2): lysine wherein the side chain amine forms the peptide linkage
EKNSSYCCELCCNPACTGCY

SEQ ID NO: 12 - protein, 13 aa, Artificial Sequence
  Synthetically generated peptide
  MOD_RES (1)..(1): allylglycine
  MOD_RES (6)..(6): allylglycine
  MOD_RES (13)..(13): AMIDATION
GCELCGNPACTGC

SEQ ID NO: 13 - protein, 13 aa, Artificial Sequence
  Synthetically generated peptide
  MOD_RES (1)..(1): allylglycine
  MOD_RES (6)..(6): allylglycine
  MOD_RES (13)..(13): AMIDATION
GCELCGNPACAGC

SEQ ID NO: 14 - protein, 14 aa, Artificial Sequence
  Synthetically generated peptide
  MOD_RES (1)..(1): allylglycine
  MOD_RES (6)..(6): allylglycine
  MOD_RES (14)..(14): AMIDATION
GCEFCGNPACTGCY

SEQ ID NO: 15 - protein, 13 aa, Artificial Sequence
  Synthetically generated peptide
  MOD_RES (1)..(1): allylglycine
  MOD_RES (4)..(4): 4-fluorophenylalanine
  MOD_RES (6)..(6): allylglycine
  MOD_RES (13)..(13): AMIDATION
GCEFCGNPACTGC

SEQ ID NO: 16 - protein, 14 aa, Artificial Sequence
  Synthetically generated peptide
  MOD_RES (1)..(1): allylglycine
  MOD_RES (4)..(4): 4-fluorophenylalanine
  MOD_RES (6)..(6): allylglycine
  MOD_RES (14)..(14): AMIDATION
GCEFCGNPACTGCY

SEQ ID NO: 17 - protein, 14 aa, Artificial Sequence
  Synthetically generated peptide
  MOD_RES (1)..(1): allylglycine
  MOD_RES (4)..(4): 4-fluorophenylalanine
  MOD_RES (6)..(6): allylglycine
  MOD_RES (14)..(14): 4-fluorophenylalanine
  MOD_RES (14)..(14): AMIDATION
GCEFCGNPACTGCF

SEQ ID NO: 18 - protein, 14 aa, Artificial Sequence
  Synthetically generated peptide
  MOD_RES (5)..(5): allylglycine
  MOD_RES (13)..(13): allylglycine
  MOD_RES (14)..(14): AMIDATION
CCELGCNPACTGGY

SEQ ID NO: 19 - protein, 13 aa, Artificial Sequence
  Synthetically generated peptide
  MOD_RES (1)..(1): allylglycine
  MOD_RES (6)..(6): allylglycine
  MOD_RES (13)..(13): AMIDATION
GCEFCGNPACTGC

SEQ ID NO: 20 - protein, 14 aa, Artificial Sequence
  Synthetically generated peptide
  MOD_RES (1)..(1): allylglycine
  MOD_RES (6)..(6): allylglycine
  MOD_RES (14)..(14): 4-fluorophenylalanine
  MOD_RES (14)..(14): AMIDATION
GCEFCGNPACTGCF

SEQ ID NO: 21 - protein, 14 aa, Artificial Sequence
  Synthetically generated peptide
  MOD_RES (4)..(4): 4-fluorophenylalanine
  MOD_RES (14)..(14): AMIDATION
CCEFCCNPACTGCY

SEQ ID NO: 22 - protein, 14 aa, Artificial Sequence
  Synthetically generated peptide
  MOD_RES (4)..(4): 4-fluorophenylalanine
  MOD_RES (14)..(14): 4-fluorophenylalanine
  MOD_RES (14)..(14): AMIDATION
CCEFCCNPACTGCF

SEQ ID NO: 23 - protein, 14 aa, Artificial Sequence
  Synthetically generated peptide
  MOD_RES (1)..(1): allylglycine
  MOD_RES (6)..(6): allylglycine
  MOD_RES (14)..(14): 4-fluorophenylalanine
  MOD_RES (14)..(14): AMIDATION
GCELCGNPACTGCF

SEQ ID NO: 24 - protein, 15 aa, Artificial Sequence
  Synthetically generated peptide
  MOD_RES (1)..(1): 4-fluorophenylalanine
  MOD_RES (2)..(2): allylglycine
  MOD_RES (7)..(7): allylglycine
  MOD_RES (15)..(15): 4-fluorophenylalanine
  MOD_RES (15)..(15): AMIDATION
FGCELCGNPACTGCF

SEQ ID NO: 25 - protein, 14 aa, Artificial Sequence
  Synthetically generated peptide
  MOD_RES (1)..(1): allylglycine
  MOD_RES (6)..(6): allylglycine
  MOD_RES (14)..(14): AMIDATION
GCELCGNPACAGCY

SEQ ID NO: 26 - protein, 14 aa, Artificial Sequence
  Synthetically generated peptide
  MOD_RES (1)..(1): allylglycine
  MOD_RES (6)..(6): allylglycine
  MOD_RES (14)..(14): AMIDATION
GCELCGNPACYGCY

SEQ ID NO: 27 - protein, 14 aa, Artificial Sequence
  Synthetically generated peptide
  MOD_RES (1)..(1): allylglycine
  MOD_RES (6)..(6): allylglycine
  MOD_RES (14)..(14): AMIDATION
GCELCGNPACFGCY

SEQ ID NO: 28 - protein, 14 aa, Artificial Sequence
  Synthetically generated peptide
  MOD_RES (1)..(1): allylglycine
  MOD_RES (6)..(6): allylglycine
  MOD_RES (11)..(11): 4-fluorophenylalanine
  MOD_RES (14)..(14): AMIDATION
GCELCGNPACFGCY

SEQ ID NO: 29 - protein, 14 aa, Artificial Sequence
  Synthetically generated peptide
  MOD_RES (1)..(1): allylglycine
  MOD_RES (6)..(6): allylglycine
  MOD_RES (14)..(14): AMIDATION
GCELCGNPACTGCL

SEQ ID NO: 30 - protein, 14 aa, Artificial Sequence
  Synthetically generated peptide
  MOD_RES (1)..(1): allylglycine
  MOD_RES (6)..(6): allylglycine
  MOD_RES (14)..(14): cyclohexylalanine
  MOD_RES (14)..(14): AMIDATION
GCELCGNPACTGCA

SEQ ID NO: 31 - protein, 14 aa, Artificial Sequence
  Synthetically generated peptide
  MOD_RES (1)..(1): allylglycine
  MOD_RES (4)..(4): cyclohexylalanine
  MOD_RES (6)..(6): allylglycine
  MOD_RES (14)..(14): AMIDATION
GCEACGNPACTGCY

SEQ ID NO: 32 - protein, 14 aa, Artificial Sequence
  Synthetically generated peptide
  MOD_RES (1)..(1): allylglycine
  MOD_RES (6)..(6): allylglycine
  MOD_RES (14)..(14): D-Tyr
  MOD_RES (14)..(14): AMIDATION
GCELCGNPACTGCY

SEQ ID NO: 33 - protein, 14 aa, Artificial Sequence
  Synthetically generated peptide
  MOD_RES (1)..(1): allylglycine
  VARIANT (2)..(2): penicillamine
  MOD_RES (6)..(6): allylglycine
  VARIANT (10)..(10): penicillamine
  MOD_RES (14)..(14): AMIDATION
GXELCGNPAXTGCY

SEQ ID NO: 34 - protein, 15 aa, Artificial Sequence
  Synthetically generated peptide
  MOD_RES (1)..(1): allylglycine
  MOD_RES (6)..(6): allylglycine
  MOD_RES (15)..(15): AMIDATION
GCELCGNPACTGCLN

SEQ ID NO: 35 - protein, 15 aa, Artificial Sequence
  Synthetically generated peptide
  MOD_RES (1)..(1): allylglycine
  MOD_RES (6)..(6): allylglycine
  MOD_RES (15)..(15): AMIDATION
GCELCGNPACTGCYN

SEQ ID NO: 36 - protein, 15 aa, Artificial Sequence
  Synthetically generated peptide
  MOD_RES (2)..(2): allylglycine
  MOD_RES (7)..(7): allylglycine
  MOD_RES (15)..(15): AMIDATION
DGCELCGNPACTGCY

SEQ ID NO: 37 - protein, 16 aa, Artificial Sequence
  Synthetically generated peptide
  MOD_RES (3)..(3): allylglycine
  MOD_RES (8)..(8): allylglycine
  MOD_RES (16)..(16): AMIDATION
IDGCELCGNPACTGCY

SEQ ID NO: 38 - protein, 14 aa, Artificial Sequence
  Synthetically generated peptide
  MOD_RES (1)..(1): allylglycine
  MOD_RES (6)..(6): allylglycine
  MOD_RES (8)..(8): hydroxyproline
  MOD_RES (14)..(14): AMIDATION
GCELCGNPACTGCY

SEQ ID NO: 39 - protein, 13 aa, Artificial Sequence
  Synthetically generated peptide
  MOD_RES (1)..(1): allylglycine
  MOD_RES (6)..(6): allylglycine
  MOD_RES (8)..(8): hydroxyproline
  MOD_RES (13)..(13): AMIDATION
GCELCGNPACTGC

SEQ ID NO: 40 - protein, 14 aa, Artificial Sequence
  Synthetically generated peptide
  MOD_RES (1)..(1): allylglycine
  VARIANT (5)..(5): penicillamine
  MOD_RES (6)..(6): allylglycine
  VARIANT (13)..(13): penicillamine
  MOD_RES (14)..(14): AMIDATION
GCELXGNPACTGXY

SEQ ID NO: 41 - protein, 14 aa, Artificial Sequence
  Synthetically generated peptide
  MOD_RES (1)..(1): allylglycine
  VARIANT (5)..(5): penicillamine
  MOD_RES (6)..(6): allylglycine
  VARIANT (13)..(13): penicillamine
  MOD_RES (14)..(14): AMIDATION
GCELXGNPACTGXY

SEQ ID NO: 42 - protein, 14 aa, Artificial Sequence
  Synthetically generated peptide
  MOD_RES (1)..(1): allylglycine
  MOD_RES (6)..(6): allylglycine
  MOD_RES (14)..(14): N-methyl tyrosine
  MOD_RES (14)..(14): AMIDATION
GCELCGNPACYGCY

SEQ ID NO: 43 - protein, 13 aa, Artificial Sequence
  Synthetically generated peptide
  MOD_RES (1)..(1): allylglycine
  MOD_RES (6)..(6): allylglycine
GCELCGNPACYGC

SEQ ID NO: 44 - protein, 14 aa, Artificial Sequence
  Synthetically generated peptide
  MOD_RES (1)..(1): allylglycine
  MOD_RES (6)..(6): allylglycine
  MOD_RES (11)..(11): cyclohexylalanine
  MOD_RES (14)..(14): AMIDATION
GCELCGNPACAGCY

SEQ ID NO: 45 - protein, 14 aa, Artificial Sequence
  Synthetically generated peptide
  MOD_RES (1)..(1): allylglycine
  MOD_RES (6)..(6): allylglycine
  MOD_RES (14)..(14): AMIDATION
GCELCGNLACTGCY

SEQ ID NO: 46 - protein, 14 aa, Artificial Sequence
  Synthetically generated peptide
  MOD_RES (1)..(1): allylglycine
  MOD_RES (6)..(6): allylglycine
  VARIANT (8)..(8): sarcosine
  MOD_RES (14)..(14): AMIDATION
GCELCGNXACTGCY

SEQ ID NO: 47 - protein, 14 aa, Artificial Sequence
  Synthetically generated peptide
  MOD_RES (1)..(1): allylglycine
  MOD_RES (6)..(6): allylglycine
  MOD_RES (14)..(14): AMIDATION
GCELCGNVACTGCY

SEQ ID NO: 48 - protein, 14 aa, Artificial Sequence
  Synthetically generated peptide
  MOD_RES (1)..(1): allylglycine
  MOD_RES (6)..(6): allylglycine
  MOD_RES (14)..(14): N-methyl tyrosine
  MOD_RES (14)..(14): AMIDATION
GCELCGNPACYGCY

SEQ ID NO: 49 - protein, 13 aa, Artificial Sequence
  Synthetically generated peptide
  MOD_RES (1)..(1): allylglycine
  MOD_RES (6)..(6): allylglycine
GCELCGLPACYGC

SEQ ID NO: 50 - protein, 13 aa, Artificial Sequence
  Synthetically generated peptide
  MOD_RES (1)..(1): allylglycine
  MOD_RES (6)..(6): allylglycine
GCDLCGNPACYGC

SEQ ID NO: 51 - protein, 13 aa, Artificial Sequence
  Synthetically generated peptide
  MOD_RES (1)..(1): allylglycine
  MOD_RES (6)..(6): allylglycine
GCSLCGNPACYGC

SEQ ID NO: 52 - protein, 13 aa, Artificial Sequence
  Synthetically generated peptide
  MOD_RES (1)..(1): allylglycine
  MOD_RES (6)..(6): allylglycine
GCTLCGNPACYGC

SEQ ID NO: 53 - protein, 14 aa, Artificial Sequence
  Synthetically generated peptide
  MOD_RES (1)..(1): allylglycine with a reduced dicarba bond
  MOD_RES (6)..(6): allylglycine with a reduced dicarba bond
  MOD_RES (14)..(14): AMIDATION
GCELCGNPACTGCY

SEQ ID NO: 54 - protein, 13 aa, Artificial Sequence
  Synthetically generated peptide
  MOD_RES (1)..(1): allylglycine
  MOD_RES (6)..(6): allylglycine
GCQLCGNPACYGC

SEQ ID NO: 55 - protein, 14 aa, Artificial Sequence
  Synthetically generated peptide
  MOD_RES (1)..(1): allylglycine
  MOD_RES (6)..(6): allylglycine
  MOD_RES (14)..(14): AMIDATION
GCELCGLPACTGCY

SEQ ID NO: 56 - protein, 13 aa, Artificial Sequence
  Synthetically generated peptide
  MOD_RES (1)..(1): N-terminus capped with pentenoic acid
  MOD_RES (5)..(5): allylglycine
  MOD_RES (13)..(13): AMIDATION
CELCGNPACYGCY

SEQ ID NO: 57 - protein, 13 aa, Artificial Sequence
  Synthetically generated peptide
  MOD_RES (6)..(6): allylglycine
  MOD_RES (13)..(13): allylglycine
CCELCGNPACYGG

SEQ ID NO: 58 - protein, 12 aa, Artificial Sequence
  Synthetically generated peptide
  MOD_RES (1)..(1): N-terminus capped with pentenoic acid
  MOD_RES (5)..(5): allylglycine
CELCGNPACYGC

SEQ ID NO: 59 - protein, 13 aa, Artificial Sequence
  Synthetically generated peptide
  MOD_RES (1)..(1): allylglycine with a reduced dicarba bond
  MOD_RES (6)..(6): allylglycine with a reduced dicarba bond
GCELCGNPACYGC

SEQ ID NO: 60 - protein, 14 aa, Artificial Sequence
  Synthetically generated peptide
  MOD_RES (1)..(1): allylglycine
  MOD_RES (6)..(6): allylglycine
  MOD_RES (14)..(14): AMIDATION
GCELCGNVACYGCY

SEQ ID NO: 61 - protein, 13 aa, Artificial Sequence
  Synthetically generated peptide
  MOD_RES (1)..(1): allylglycine
  MOD_RES (6)..(6): allylglycine
GCELCGNVACYGC

SEQ ID NO: 62 - protein, 14 aa, Artificial Sequence
  Synthetically generated peptide
  VARIANT (2)..(2): cystathionine
  MOD_RES (14)..(14): AMIDATION
CXELCCNPACYGCY

SEQ ID NO: 63 - protein, 14 aa, Artificial Sequence
  Synthetically generated peptide
  VARIANT (1)..(1): cystathionine
  MOD_RES (14)..(14): AMIDATION
XCELCCNPACYGCY

SEQ ID NO: 64 - protein, 14 aa, Artificial Sequence
  Synthetically generated peptide
  VARIANT (1)..(1): cystathionine
XCELCCNPACYGCY

SEQ ID NO: 65 - protein, 14 aa, Artificial Sequence
  Synthetically generated peptide
  VARIANT (2)..(2): cystathionine
  MOD_RES (14)..(14): AMIDATION
CXELCCNVACYGCY

SEQ ID NO: 66 - protein, 14 aa, Artificial Sequence
  Synthetically generated peptide
  VARIANT (2)..(2): cystathionine
  MOD_RES (14)..(14): AMIDATION
CXELCCNVACTGCY

SEQ ID NO: 67 - protein, 14 aa, Artificial Sequence
  Synthetically generated peptide
  MOD_RES (1)..(1): acetylated N-terminus
  MOD_RES (2)..(2): cystathionine
  MOD_RES (14)..(14): AMIDATION
CXELCCNVACTGCY

SEQ ID NO: 68 - protein, 14 aa, Artificial Sequence
  Synthetically generated peptide
  MOD_RES (1)..(1): acetylated N-terminus
  VARIANT (2)..(2): cystathionine
  MOD_RES (14)..(14): ACETYLATION
CXELCCNPACYGCY

SEQ ID NO: 69 - protein, 13 aa, Artificial Sequence
  Synthetically generated peptide
  MOD_RES (1)..(1): acetylated N-terminus
  VARIANT (2)..(2): cystathionine
CXELCCNVACYGC

SEQ ID NO: 70 - protein, 13 aa, Artificial Sequence
  Synthetically generated peptide
  VARIANT (2)..(2): cystathionine
CXELCCNVACYGC

SEQ ID NO: 71 - protein, 13 aa, Artificial Sequence
  Synthetically generated peptide
  MOD_RES (1)..(1): acetylated N-terminus
  VARIANT (2)..(2): cystathionine
CXELCCNPACYGC

SEQ ID NO: 72 - protein, 12 aa, Artificial Sequence
  Synthetically generated peptide
  VARIANT (9)..(9): cystathionine
CCELCNVAXYGC

SEQ ID NO: 73 - protein, 14 aa, Artificial Sequence
  Synthetically generated peptide
  VARIANT (10)..(10): cystathionine
  MOD_RES (14)..(14): AMIDATION
CCELCCNVAXYGCY

SEQ ID NO: 74 - protein, 14 aa, Artificial Sequence
  Synthetically generated peptide
  VARIANT (10)..(10): cystathionine
  MOD_RES (14)..(14): AMIDATION
CCELCCNVAXTGCY

SEQ ID NO: 75 - protein, 13 aa, Artificial Sequence
  Synthetically generated peptide
  VARIANT (6)..(6): cystathionine
CCELCXNVACYGC

SEQ ID NO: 76 - protein, 14 aa, Artificial Sequence
  Synthetically generated peptide
  VARIANT (6)..(6): cystathionine
  MOD_RES (14)..(14): AMIDATION
CCELCXNVACYGCY

SEQ ID NO: 77 - protein, 14 aa, Artificial Sequence
  Synthetically generated peptide
  VARIANT (6)..(6): cystathionine
  MOD_RES (14)..(14): AMIDATION
CCELCXNVACTGCY

SEQ ID NO: 78 - protein, 13 aa, Artificial Sequence
  Synthetically generated peptide
  MOD_RES (1)..(1): N-terminus capped with 4-Mepip (1-methyl-piperidine-4-carboxylic acid)
  VARIANT (2)..(2): cystathionine
CXELCCNVACYGC

SEQ ID NO: 79 - protein, 13 aa, Artificial Sequence
  Synthetically generated peptide
  VARIANT (2)..(2): cystathionine
CXELCCNVACTGC

SEQ ID NO: 80 - protein, 13 aa, Artificial Sequence
  Synthetically generated peptide
  VARIANT (2)..(2): cystathionine
  MOD_RES (13)..(13): AMIDATION
CXELCCNVACTGC

SEQ ID NO: 81 - protein, 13 aa, Artificial Sequence
  Synthetically generated peptide
  VARIANT (2)..(2): cystathionine
CXELCCNVACFGC

SEQ ID NO: 82 - protein, 14 aa, Artificial Sequence
  Synthetically generated peptide
  MOD_RES (1)..(1): allylglycine
  MOD_RES (2)..(2): allylglycine
  MOD_RES (5)..(5): allylglycine
  MOD_RES (6)..(6): allylglycine
  MOD_RES (10)..(10): allylglycine
  MOD_RES (13)..(13): allylglycine
GGELGGNPAGTGGY

SEQ ID NO: 83 - protein, 14 aa, Artificial Sequence
  Synthetically generated peptide
  VARIANT (2)..(2): cystathionine
  MOD_RES (14)..(14): AMIDATION
CXELCCNAACTGCY

SEQ ID NO: 84 - protein, 14 aa, Artificial Sequence
  Synthetically generated peptide
  VARIANT (6)..(6): di-aminopropionic acid
  MOD_RES (14)..(14): AMIDATION
DCELCXNVACTGCY

SEQ ID NO: 85 - protein, 14 aa, Artificial Sequence
  Synthetically generated peptide
  VARIANT (2)..(2): cystathionine
  MOD_RES (14)..(14): AMIDATION
CXELCCNVACSGCY

SEQ ID NO: 86 - protein, 13 aa, Artificial Sequence
  Synthetically generated peptide
  VARIANT (1)..(1): cystathionine
  MOD_RES (5)..(5): allylglycine
  MOD_RES (13)..(13): AMIDATION
XELCGNVACTGCY

SEQ ID NO: 87 - protein, 14 aa, Artificial Sequence
  Synthetically generated peptide
  MOD_RES (1)..(1): allylglycine
  MOD_RES (6)..(6): allylglycine
  MOD_RES (14)..(14): AMIDATION
GCELCGNVACTGCY

SEQ ID NO: 88 - protein, 14 aa, Artificial Sequence
  Synthetically generated peptide
  MOD_RES (1)..(1): allylglycine
  MOD_RES (6)..(6): allylglycine
  MOD_RES (14)..(14): AMIDATION
GCELCGNPACTGCY

SEQ ID NO: 89 - protein, 13 aa, Artificial Sequence
  Synthetically generated peptide
  VARIANT (1)..(1): cystathionine
XCELCCNVACTGC

SEQ ID NO: 90 - protein, 14 aa, Artificial Sequence
  Synthetically generated peptide
  VARIANT (1)..(1): cystathionine
  MOD_RES (14)..(14): AMIDATION
XCELCCNVACTGCY

SEQ ID NO: 91 - protein, 14 aa, Artificial Sequence
  Synthetically generated peptide
  VARIANT (1)..(1): cystathionine
  MOD_RES (14)..(14): AMIDATION
XCELCCNVACYGCY

SEQ ID NO: 92 - protein, 13 aa, Artificial Sequence
  Synthetically generated peptide
  misc_feature (10)..(10): Xaa can be any naturally occurring amino acid
  VARIANT (13)..(13): cystathionine
CCELCCNVAXYGC

SEQ ID NO: 93 - protein, 21 aa, Artificial Sequence
  Synthetically generated peptide
  VARIANT (1)..(1): Xaa1 is glutamic acid wherein the side chain carboxylic acid forms the peptide linkage or is absent
  VARIANT (2)..(2): Xaa1 is lysine wherein the side chain amine forms the peptide linkage or is absent
  VARIANT (3)..(3): Xaa3 is Asn or is absent
  VARIANT (4)..(4): Xaa4 is Ser or is absent
  VARIANT (5)..(5): Xaa5 is Ser, Asn, Ile, or is absent
  VARIANT (6)..(6): Xaa6 is Tyr, Asp, 4-fluorophenylalanine ((4-F)Phe), or is absent
  VARIANT (7)..(7): Xaa7 is Cys, cystathionine (Cth), allylglycine (Ag), allylglycine with a reduced dicarba bond (Hag), or Asp
  VARIANT (8)..(8): Xaa8 is Cys, cystathionine (Cth), penicillamine (Pen), or allylglycine (Ag)
  VARIANT (9)..(9): Xaa9 is Glu, Asp, Ser, Thr, or Gln
  VARIANT (10)..(10): Xaa10 is Leu, cyclohexylalanine (Cha), Phe, or 4-fluorophenylalanine ((4-F)Phe)
  VARIANT (12)..(12): Xaa12 is Cys, allylglycine (Ag), Hag, or Val
  VARIANT (14)..(14): Xaa14 is Pro, Val, sarcosine (Sar), Leu, or Hydroxyproline (OH-Pro)
  VARIANT (17)..(17): Xaa17 is Tyr, Thr, cyclohexylalanine (Cha), 4-fluorophenylalanine ((4-F)Phe), Phe, or Ala
  VARIANT (20)..(20): Xaa20 is Tyr, Leu, 4-fluorophenylalanine ((4-F)Phe), cyclohexylalanine (Cha), D-Tyr, N-Methyl Tyr (Nme-Tyr) or is absent
  VARIANT (21)..(21): Xaa21 is absent or Asnt
XXXXXXXXXXCXNXACXGCXX

SEQ ID NO: 94 - protein, 14 aa, Artificial Sequence
  Synthetically generated peptide
CCELCCNPACTGCY